European Patent Specification EP 3 820 892 B1, published January 3, 2024. Title: ANTIBODIES HAVING SPECIFICITY FOR THE ORF2I PROTEIN OF HEPATITIS E VIRUS AND USES THEREOF FOR DIAGNOSTIC PURPOSES. Applicant: Inserm. The sequence listing filed with the application follows.

SEQUENCE LISTING (4 sequences)

SEQ ID NO: 1 - protein, 647 aa, Hepatitis E virus
LPMLPAPPAGQPSGRRRGRRSGGAGGGFWGDRVDSQPFALPYIHPTNPFAADIVSQSGAGTRPRQPPRPLGSAWRDQSQRPSAAPRRRSAPAGAAPLTAVSPAPDTAPVPDVDSRGAILRRQYNLSTSPLTSSVASGTNLVLYAAPLNPLLPLQDGTNTHIMATEASNYAQYRVVRATIRYRPLVPNAVGGYAISISFWPQTTTTPTSVDMNSITSTDVRILVQPGIASELVIPSERLHYRNQGWRSVETTGVAEEEATSGLVMLCIHGSPVNSYTNTPYTGALGLLDFALELEFRNLTPGNTNTRVSRYTSTARHRLRRGADGTAELTTTAATRFMKDLHFTGTNGVGEVGRGIALTLFNLADTLLGGLPTELISSAGGQLFYSRPVVSANGEPTVKLYTSVENAQQDKGITIPHDIDLGDSRVVIQDYDNQHEQDRPTPSPAPSRPFSVLRANDVLWLSLTAAEYDQATYGSSTNPMYVSDTVTFVNVATGAQAVARSLDWSKVTLDGRPLTTIQQYSKTFYVLPLRGKLSFWEAGTTRAGYPYNYNTTASDQILIENAAGHRVAISTYTTSLGAGPASISAVGVLAPHSALAVLEDTVDYPARAHTFDDFCPECRTLGLQGCAFQSTIAELQRLKTEVGKTRES

SEQ ID NO: 2 - protein, 627 aa, Hepatitis E virus
SGGAGGGFWGDRVDSQPFALPYIHPTNPFAADIVSQSGAGTRPRQPPRPLGSAWRDQSQRPSAAPRRRSAPAGAAPLTAVSPAPDTAPVPDVDSRGAILRRQYNLSTSPLTSSVASGTNLVLYAAPLNPLLPLQDGTNTHIMATEASNYAQYRVVRATIRYRPLVPNAVGGYAISISFWPQTTTTPTSVDMNSITSTDVRILVQPGIASELVIPSERLHYRNQGWRSVETTGVAEEEATSGLVMLCIHGSPVNSYTNTPYTGALGLLDFALELEFRNLTPGNTNTRVSRYTSTARHRLRRGADGTAELTTTAATRFMKDLHFTGTNGVGEVGRGIALTLFNLADTLLGGLPTELISSAGGQLFYSRPVVSANGEPTVKLYTSVENAQQDKGITIPHDIDLGDSRVVIQDYDNQHEQDRPTPSPAPSRPFSVLRANDVLWLSLTAAEYDQATYGSSTNPMYVSDTVTFVNVATGAQAVARSLDWSKVTLDGRPLTTIQQYSKTFYVLPLRGKLSFWEAGTTRAGYPYNYNTTASDQILIENAAGHRVAISTYTTSLGAGPASISAVGVLAPHSALAVLEDTVDYPARAHTFDDFCPECRTLGLQGCAFQSTIAELQRLKTEVGKTRES

SEQ ID NO: 3 - protein, 559 aa, Hepatitis E virus
SAPAGAAPLTAVSPAPDTAPVPDVDSRGAILRRQYNLSTSPLTSSVASGTNLVLYAAPLNPLLPLQDGTNTHIMATEASNYAQYRVVRATIRYRPLVPNAVGGYAISISFWPQTTTTPTSVDMNSITSTDVRILVQPGIASELVIPSERLHYRNQGWRSVETTGVAEEEATSGLVMLCIHGSPVNSYTNTPYTGALGLLDFALELEFRNLTPGNTNTRVSRYTSTARHRLRRGADGTAELTTTAATRFMKDLHFTGTNGVGEVGRGIALTLFNLADTLLGGLPTELISSAGGQLFYSRPVVSANGEPTVKLYTSVENAQQDKGITIPHDIDLGDSRVVIQDYDNQHEQDRPTPSPAPSRPFSVLRANDVLWLSLTAAEYDQATYGSSTNPMYVSDTVTFVNVATGAQAVARSLDWSKVTLDGRPLTTIQQYSKTFYVLPLRGKLSFWEAGTTRAGYPYNYNTTASDQILIENAAGHRVAISTYTTSLGAGPASISAVGVLAPHSALAVLEDTVDYPARAHTFDDFCPECRTLGLQGCAFQSTIAELQRLKTEVGKTRES

SEQ ID NO: 4 - protein, 14 aa, Hepatitis E virus
GQPSGRRRGRRSGG